European Patent Application EP 4 471 056 A1, published December 4, 2024. Title: ANTI-DKK1 ANTIBODY, PHARMACEUTICAL COMPOSITION THEREOF, AND USE THEREOF. Applicant: SHANGHAI JUNSHI BIOSCIENCES CO., LTD. The sequence listing filed with the application follows.

SEQUENCE LISTING (113 sequences)

SEQ ID NO: 1 - protein, 5 aa, synthetic construct
EYTMH

SEQ ID NO: 2 - protein, 17 aa, synthetic construct
VIDPSNGDTSYNQKFKG

SEQ ID NO: 3 - protein, 8 aa, synthetic construct
TTGPWFAS

SEQ ID NO: 4 - protein, 11 aa, synthetic construct
RASQDISNYLN

SEQ ID NO: 5 - protein, 7 aa, synthetic construct
YKSRLHS

SEQ ID NO: 6 - protein, 9 aa, synthetic construct
QQVHTLPPT

SEQ ID NO: 7 - protein, 5 aa, synthetic construct
ENTMH

SEQ ID NO: 8 - protein, 17 aa, synthetic construct
GINPHKGGTSYNQKFKG

SEQ ID NO: 9 - protein, 8 aa, synthetic construct
DWLGAMDY

SEQ ID NO: 10 - protein, 11 aa, synthetic construct
ITSTDIDDDMN

SEQ ID NO: 11 - protein, 7 aa, synthetic construct
EGNTLRP

SEQ ID NO: 12 - protein, 9 aa, synthetic construct
LQSDNLPYT

SEQ ID NO: 13 - protein, 5 aa, synthetic construct
SYNML

SEQ ID NO: 14 - protein, 17 aa, synthetic construct
VIFPGNGDTSYNPKFKG

SEQ ID NO: 15 - protein, 8 aa, synthetic construct
DGYPSMDY

SEQ ID NO: 16 - protein, 11 aa, synthetic construct
ITSTDIDDDMN

SEQ ID NO: 17 - protein, 7 aa, synthetic construct
EGNSLRP

SEQ ID NO: 18 - protein, 9 aa, synthetic construct
LQFNNMPLT

SEQ ID NO: 19 - protein, 7 aa, synthetic construct
TSGMGVG

SEQ ID NO: 20 - protein, 16 aa, synthetic construct
HIWWDDVKRYNPALKS

SEQ ID NO: 21 - protein, 10 aa, synthetic construct
IARSPTGFAY

SEQ ID NO: 22 - protein, 10 aa, synthetic construct
SASSSVSYMY

SEQ ID NO: 23 - protein, 7 aa, synthetic construct
DTSNLAS

SEQ ID NO: 24 - protein, 11 aa, synthetic construct
QQWSSYPPALT

SEQ ID NO: 25 - protein, 5 aa, synthetic construct
AFDVH

SEQ ID NO: 26 - protein, 16 aa, synthetic construct
VIWIGGTTDYNGAFIS

SEQ ID NO: 27 - protein, 10 aa, synthetic construct
KRGNYYNMDY

SEQ ID NO: 28 - protein, 14 aa, synthetic construct
RSSTGTVTTTNYAN

SEQ ID NO: 29 - protein, 7 aa, synthetic construct
GTNNRAP

SEQ ID NO: 30 - protein, 9 aa, synthetic construct
ALWYSNHWV

SEQ ID NO: 31 - protein, 5 aa, synthetic construct
NHGMN

SEQ ID NO: 32 - protein, 17 aa, synthetic construct
WINTNTGEPTYADDFKG

SEQ ID NO: 33 - protein, 13 aa, synthetic construct
RGYGFPYYYTMDY

SEQ ID NO: 34 - protein, 14 aa, synthetic construct
RSSTGAVTTRNYAN

SEQ ID NO: 35 - protein, 7 aa, synthetic construct
GTKNRAP

SEQ ID NO: 36 - protein, 9 aa, synthetic construct
ALWYSNRLV

SEQ ID NO: 37 - protein, 136 aa, synthetic construct
MGWSWIFLFLLSGTAGVLSEVQLQQSGPELVKPGASVRISCKTSGYTFTEYTMHWVKQSHGKSLEWIGVIDPSNGDTSYNQKFKGRATLTVDKSSSTAYMDLRSLTSEDSALYYCSSTTGPWFACWGQGTLVTVSA

SEQ ID NO: 38 - protein, 126 aa, synthetic construct
MSSAQFLGLLLLCFQGTRCDIQMTQTTSSLSASLGDRVTINCRASQDISNYLNWYQQKPDGTVKLLIYYKSRLHSGVPTRFSGSGSGTDFSLTISNLVQEDIATYFCQQVHTLPPTFGGGTKLEIK

SEQ ID NO: 39 - protein, 136 aa, synthetic construct
MGWSWIFLFLLSGTAGVLSEVQLQQSGPELVKPGASVKIFCKTSGYTFTENTMHWVKQTHGKSLEWIGGINPHKGGTSYNQKFKGKATLTVDKSSSTACMELRSLTSEDSTVYYCARDWLGAMDYWGQGTSVTVSP

SEQ ID NO: 40 - protein, 127 aa, synthetic construct
MFSLALLLSLLLLCVSDSRAETTVTQSPASLSMAIGEKVTIRCITSTDIDDDMNWYQQKPGEPPKLLISEGNTLRPGVPSRFSSSGYGTDFVFTIENMLSEDVADYYCLQSDNLPYTFGGGTKLEIK

SEQ ID NO: 41 - protein, 136 aa, synthetic construct
MGWNCFILFLVATATGVHSQVQLQQPGAELVKPGASVKMSCKASGYTFTSYNMLWVKQTPGQGLEWIGVIFPGNGDTSYNPKFKGKAALTADKSSSTAYMQLSSLTSEDSAVYYCARDGYPSMDYWGQGTSVTVSS

SEQ ID NO: 42 - protein, 127 aa, synthetic construct
MLSLAPLLSLLLLCVSDSRAETIVTQSPASLSVATGEKVTIRCITSTDIDDDMNWYQQKPGEPPKLLISEGNSLRPGVPSRFSSSGYGTDFVFTIENTLSEDVADYYCLQFNNMPLTFGAGTKLELK

SEQ ID NO: 43 - protein, 134 aa, synthetic construct
MGRLTSSFLLLIVPAYVLSQVTLKESGPGILQPSQTLSLTCSFSGFSLSTSGMGVGWIRQPSGKGLEWLAHIWWDDVKRYNPALKSRLTISKDTSSSQVFLKIASVDTTDTASYYCSRIARSPTGFAYWGQGTL

SEQ ID NO: 44 - protein, 130 aa, synthetic construct
MDFQVQIFSFLLISASVILSRGQIVLTQSPVIMSASPGEKVTMTCSASSSVSYMYWYQQKPGSSPRLLIYDTSNLASGVPVRFSGSGSGTSYSLTISRMEAEDAATYYCQQWSSYPPALTFGAGTKLELK

SEQ ID NO: 45 - protein, 137 aa, synthetic construct
MAVLGLLFCLVTFPSCVLSQVQLKQSGPGLVQPSQSLSITCTVSGFSLTAFDVHWVRQSPGKGLEWLGVIWIGGTTDYNGAFISRLSISKDNSKSQVFFKMNSLQAKDTAIYYCARKRGNYYNMDYWGQGTSVTVAS

SEQ ID NO: 46 - protein, 128 aa, synthetic construct
MAWISLILSLLALSSGAISQAVVTQESALTTSPGETVTLTCRSSTGTVTTTNYANWVQEKPDHLFTGLIGGTNNRAPGVPARFSGSLIGDKAALTITGAQTEDEAIYFCALWYSNHWVFGGGTKLTVL

SEQ ID NO: 47 - protein, 141 aa, synthetic construct
MAWVWTLLFLMAAAQSAQAQIQLVQSGPELKKPGETVKISCKASGYTFTNHGMNWVKQAPGKGLKWMGWINTNTGEPTYADDFKGRFAFSLETSASTAYLQINNLKNEDTATYFCARRGYGFPYYYTMDYWGQGTSVTVSS

SEQ ID NO: 48 - protein, 128 aa, synthetic construct
MAWISLILSLLALSSGAISQAVVTQESALTTSPGETVTLTCRSSTGAVTTRNYANWVQEKADHLLTGLIGGTKNRAPGVPARFSGSLIGDKAALTITGAQTEDEAKYFCALWYSNRLVFGGGTKLTVL

SEQ ID NO: 49 - protein, 117 aa, synthetic construct
EVQLLQSAAEVKRPGESLRISCKTSGYTFTEYTMHWVRQMPGKELEWMGVIDPSNGDTSYNQKFKGHVTISADKSSSTAYLQWSSLKASDAAMYYCSSTTGPWFASWGQGTLVTVSS

SEQ ID NO: 50 - protein, 117 aa, synthetic construct
QVQLVQSGAEVKKPGASVKVSCKASGYTFTEYTMHWVRQAPGQGLEWMGVIDPSNGDTSYNQKFKGRVTLTVDKSTSTAYMELRSLRSDDTAVYYCARTTGPWFASWGQGTLVTVSS

SEQ ID NO: 51 - protein, 117 aa, synthetic construct
QVQLVQSGAEVKKPGSSVKVSCKASGYTFTEYTMHWVRQAPGQGLEWMGVIDPSNGDTSYNQKFKGRVTITADKSTSTAYMELSSLRSEDTAVYYCSSTTGPWFASWGQGTLVTVSS

SEQ ID NO: 52 - protein, 117 aa, synthetic construct
QVQLVQSGAEVKKPGASVKVSCKASGYTFTEYTMHWVRQAPGQRLEWMGVIDPSNGDTSYNQKFKGRVTITVDKSSSTAYMELSSLRSEDTAVYYCSSTTGPWFASWGQGTLVTVSS

SEQ ID NO: 53 - protein, 117 aa, synthetic construct
QVQLVQSGAEVKKPGASVKVSCKASGYTFTEYTMHWVRQAPGQRLEWMGVIDPSNGDTSYNQKFKGRVTLTVDKSSSTAYMELSSLRSEDTAVYYCARTTGPWFASWGQGTLVTVSS

SEQ ID NO: 54 - protein, 107 aa, synthetic construct
DIQMTQSPSSLSASVGDRVTITCRASQDISNYLNWYQQKPGKAPKLLIYYKSRLHSGVPSRFSGSGSGTDFTFTISSLQPEDIATYYCQQVHTLPPTFGQGTKLEIK

SEQ ID NO: 55 - protein, 107 aa, synthetic construct
DIQMTQSPSSLSASVGDRVTITCRASQDISNYLNWYQQKPGKAPKLLIYYKSRLHSGVPSRFSGSGSGTDFTLTISSLQPEDFATYYCQQVHTLPPTFGQGTKLEIK

SEQ ID NO: 56 - protein, 107 aa, synthetic construct
EIVMTQSPPTLSLSPGERVTLSCRASQDISNYLNWYQQKPGQAPRLLIYYKSRLHSGIPARFSGSGSGTDFTLTISSLQPEDFAVYYCQQVHTLPPTFGQGTKLEIK

SEQ ID NO: 57 - protein, 107 aa, synthetic construct
DIQMTQSPSSLSASVGDRVTITCRASQDISNYLNWYQQKPGKAPKLLIYYKSRLHSGVPSRFSGSGSGTDFTFTISSLQPEDIATYFCQQVHTLPPTFGQGTKLEIK

SEQ ID NO: 58 - protein, 117 aa, synthetic construct
EVQLLQSAAEVKRPGESLRISCKTSGYSFTENTMHWVRQMPGKELEWMGGINPHKGGTSYNQKFKGHVTISVDKSSSTAYLQWSSLKASDAAMYYCARDWLGAMDYWGQGTLVTVSS

SEQ ID NO: 59 - protein, 117 aa, synthetic construct
EVQLLQSAAEVKRPGESLRISCKTSGYTFTENTMHWVRQMPGKELEWMGGINPHKGGTSYNQKFKGHVTISADKSSSTAYLQWSSLKASDAAMYYCARDWLGAMDYWGQGTLVTVSS

SEQ ID NO: 60 - protein, 117 aa, synthetic construct
EVQLLQSAAEVKRPGESLRISCKTSGYTFTENTMHWVRQMPGKELEWMGGINPHKGGTSYNQKFKGHVTLSVDKSSSTAYLQWSSLKASDAAMYYCARDWLGAMDYWGQGTLVTVSS

SEQ ID NO: 61 - protein, 117 aa, synthetic construct
QVQLVQSGAEVKKPGASVKVSCKASGYTFTENTMHWVRQAPGQGLEWMGGINPHKGGTSYNQKFKGRVTLTVDKSSSTAYMELSRLRSDDTAVYYCARDWLGAMDYWGQGTLVTVSS

SEQ ID NO: 62 - protein, 117 aa, synthetic construct
QVQLVQSGAEVKKPGSSVKVSCKASGYTFTENTMHWVRQAPGQGLEWMGGINPHKGGTSYNQKFKGRVTITVDKSTSTAYMELSSLRSEDTAVYYCARDWLGAMDYWGQGTLVTVSS

SEQ ID NO: 63 - protein, 107 aa, synthetic construct
DIQLTQSPSSLSASVGDRVTITCITSTDIDDDMNWYRQKPGKVPKLLISEGNTLRPGVPSRFSGSGSGTDFTLTISSLQPEDVATYYCLQSDNLPYTFGQGTKLEIK

SEQ ID NO: 64 - protein, 107 aa, synthetic construct
DIQVTQSPSSLSASVGDRVTITCITSTDIDDDMNWYQQKPGKAPKLLISEGNTLRPGVPSRFSGSGSGTDFTFTISSLQPEDIATYYCLQSDNLPYTFGQGTKLEIK

SEQ ID NO: 65 - protein, 107 aa, synthetic construct
DIVLTQSPASLAVSPGQRATITCITSTDIDDDMNWYQQKPGQPPKLLISEGNTLRPGVPARFSSSGSGTDFTLTINPVEANDTANYYCLQSDNLPYTFGQGTKLEIK

SEQ ID NO: 66 - protein, 107 aa, synthetic construct
DTVLTQSPASLAVSPGQRATITCITSTDIDDDMNWYQQKPGQPPKLLISEGNTLRPGVPARFSSSGSGTDFTLTINPVEANDTANYYCLQSDNLPYTFGQGTKLEIK

SEQ ID NO: 67 - protein, 107 aa, synthetic construct
DIVLTQSPASLAVSPGQRATITCITSTDIDDDMNWYQQKPGQPPKLLISEGNTLRPGVPARFSSSGSGTDFTLTINPVEANDVANYYCLQSDNLPYTFGQGTKLEIK

SEQ ID NO: 68 - protein, 117 aa, synthetic construct
QVQLVQSGAEVKKPGASVKVSCKASGYTFTSYNMLWVRQAPGQRLEWMGVIFPGNGDTSYNPKFKGRVTITADKSSSTAYMELSSLRSEDTAVYYCARDGYPSMDYWGQGTLVTVSS

SEQ ID NO: 69 - protein, 117 aa, synthetic construct
QVQLVQSGAEVKKPGASVKVSCKASGYTFTSYNMLWVRQAPGQRLEWMGVIFPGNGDTSYNPKFKGRVTLTADKSSSTAYMELSSLRSEDTAVYYCARDGYPSMDYWGQGTLVTVSS

SEQ ID NO: 70 - protein, 117 aa, synthetic construct
QVQLVQSGAEVKKPGSSVKVSCKASGYTFSSYNMLWVRQAPGQGLEWMGVIFPGNGDTSYNPKFKGRVTITADKSTSTAYMELSSLRSEDTAVYYCARDGYPSMDYWGQGTLVTVSS

SEQ ID NO: 71 - protein, 117 aa, synthetic construct
QVQLVQSGAEVKKPGSSVKVSCKASGYTFTSYNMLWVRQAPGQGLEWMGVIFPGNGDTSYNPKFKGRVTITADKSTSTAYMELSSLRSEDTAVYYCARDGYPSMDYWGQGTLVTVSS

SEQ ID NO: 72 - protein, 117 aa, synthetic construct
QVQLVQSGAEVKKPGSSVKVSCKASGYTFTSYNMLWVRQAPGQGLEWMGVIFPGNGDTSYNPKFKGRVTLTADKSSSTAYMELSSLRSEDTAVYYCARDGYPSMDYWGQGTLVTVSS

SEQ ID NO: 73 - protein, 117 aa, synthetic construct
QVQLVQSGAEVKKPGASVKVSCKASGYTFTSYNMLWVRQAPGQRLEWMGVIFPGNADTSYNPKFKGRVTLTADKSSSTAYMELSSLRSEDTAVYYCARDGYPSMDYWGQGTLVTVSS

SEQ ID NO: 74 - protein, 107 aa, synthetic construct
DIQMTQSPSSVSASVGDRVTITCITSTDIDDDMNWYQQKPGKAPKLLISEGNSLRPGVPSRFSGSGSGTDFTLTISSLQPEDFATYYCLQFNNMPLTFGQGTKLEIK

SEQ ID NO: 75 - protein, 107 aa, synthetic construct
DIQLTQSPSFLSASVGDRVTITCITSTDIDDDMNWYQQKPGKAPKLLISEGNSLRPGVPSRFSSSGSGTEFTLTISSLQPEDFATYYCLQFNNMPLTFGQGTKLEIK

SEQ ID NO: 76 - protein, 107 aa, synthetic construct
DTQLTQSPSFLSASVGDRVTITCITSTDIDDDMNWYQQKPGKAPKLLISEGNSLRPGVPSRFSSSGSGTEFTLTISSLQPEDFATYYCLQFNNMPLTFGQGTKLEIK

SEQ ID NO: 77 - protein, 107 aa, synthetic construct
EIVLTQSPDFQSVTPKEKVTITCITSTDIDDDMNWYQQKPDQSPKLLISEGNSLRPGVPSRFSSSGSGTDFTLTINSLEAEDAATYYCLQFNNMPLTFGQGTKLEIK

SEQ ID NO: 78 - protein, 8 aa, synthetic construct
TTGPWFAC

SEQ ID NO: 79 - protein, 444 aa, synthetic construct
EVQLLQSAAEVKRPGESLRISCKTSGYTFTEYTMHWVRQMPGKELEWMGVIDPSNGDTSYNQKFKGHVTISADKSSSTAYLQWSSLKASDAAMYYCSSTTGPWFASWGQGTLVTVSSASTKGPSVFPLAPCSRSTSESTAALGCLVKDYFPEPVTVSWNSGALTSGVHTFPAVLQSSGLYSLSSVVTVPSSSLGTKTYTCNVDHKPSNTKVDKRVESKYGPPCPPCPAPEFLGGPSVFLFPPKPKDTLMISRTPEVTCVVVDVSQEDPEVQFNWYVDGVEVHNAKTKPREEQFNSTYRVVSVLTVLHQDWLNGKEYKCKVSNKGLPSSIEKTISKAKGQPREPQVYTLPPSQEEMTKNQVSLTCLVKGFYPSDIAVEWESNGQPENNYKTTPPVLDSDGSFFLYSRLTVDKSRWQEGNVFSCSVMHEALHNHYTQKSLSLSLGK

SEQ ID NO: 80 - protein, 444 aa, synthetic construct
QVQLVQSGAEVKKPGASVKVSCKASGYTFTEYTMHWVRQAPGQGLEWMGVIDPSNGDTSYNQKFKGRVTLTVDKSTSTAYMELRSLRSDDTAVYYCARTTGPWFASWGQGTLVTVSSASTKGPSVFPLAPCSRSTSESTAALGCLVKDYFPEPVTVSWNSGALTSGVHTFPAVLQSSGLYSLSSVVTVPSSSLGTKTYTCNVDHKPSNTKVDKRVESKYGPPCPPCPAPEFLGGPSVFLFPPKPKDTLMISRTPEVTCVVVDVSQEDPEVQFNWYVDGVEVHNAKTKPREEQFNSTYRVVSVLTVLHQDWLNGKEYKCKVSNKGLPSSIEKTISKAKGQPREPQVYTLPPSQEEMTKNQVSLTCLVKGFYPSDIAVEWESNGQPENNYKTTPPVLDSDGSFFLYSRLTVDKSRWQEGNVFSCSVMHEALHNHYTQKSLSLSLGK

SEQ ID NO: 81 - protein, 444 aa, synthetic construct
QVQLVQSGAEVKKPGSSVKVSCKASGYTFTEYTMHWVRQAPGQGLEWMGVIDPSNGDTSYNQKFKGRVTITADKSTSTAYMELSSLRSEDTAVYYCSSTTGPWFASWGQGTLVTVSSASTKGPSVFPLAPCSRSTSESTAALGCLVKDYFPEPVTVSWNSGALTSGVHTFPAVLQSSGLYSLSSVVTVPSSSLGTKTYTCNVDHKPSNTKVDKRVESKYGPPCPPCPAPEFLGGPSVFLFPPKPKDTLMISRTPEVTCVVVDVSQEDPEVQFNWYVDGVEVHNAKTKPREEQFNSTYRVVSVLTVLHQDWLNGKEYKCKVSNKGLPSSIEKTISKAKGQPREPQVYTLPPSQEEMTKNQVSLTCLVKGFYPSDIAVEWESNGQPENNYKTTPPVLDSDGSFFLYSRLTVDKSRWQEGNVFSCSVMHEALHNHYTQKSLSLSLGK

SEQ ID NO: 82 - protein, 444 aa, synthetic construct
QVQLVQSGAEVKKPGASVKVSCKASGYTFTEYTMHWVRQAPGQRLEWMGVIDPSNGDTSYNQKFKGRVTITVDKSSSTAYMELSSLRSEDTAVYYCSSTTGPWFASWGQGTLVTVSSASTKGPSVFPLAPCSRSTSESTAALGCLVKDYFPEPVTVSWNSGALTSGVHTFPAVLQSSGLYSLSSVVTVPSSSLGTKTYTCNVDHKPSNTKVDKRVESKYGPPCPPCPAPEFLGGPSVFLFPPKPKDTLMISRTPEVTCVVVDVSQEDPEVQFNWYVDGVEVHNAKTKPREEQFNSTYRVVSVLTVLHQDWLNGKEYKCKVSNKGLPSSIEKTISKAKGQPREPQVYTLPPSQEEMTKNQVSLTCLVKGFYPSDIAVEWESNGQPENNYKTTPPVLDSDGSFFLYSRLTVDKSRWQEGNVFSCSVMHEALHNHYTQKSLSLSLGK

SEQ ID NO: 83 - protein, 444 aa, synthetic construct
QVQLVQSGAEVKKPGASVKVSCKASGYTFTEYTMHWVRQAPGQRLEWMGVIDPSNGDTSYNQKFKGRVTLTVDKSSSTAYMELSSLRSEDTAVYYCARTTGPWFASWGQGTLVTVSSASTKGPSVFPLAPCSRSTSESTAALGCLVKDYFPEPVTVSWNSGALTSGVHTFPAVLQSSGLYSLSSVVTVPSSSLGTKTYTCNVDHKPSNTKVDKRVESKYGPPCPPCPAPEFLGGPSVFLFPPKPKDTLMISRTPEVTCVVVDVSQEDPEVQFNWYVDGVEVHNAKTKPREEQFNSTYRVVSVLTVLHQDWLNGKEYKCKVSNKGLPSSIEKTISKAKGQPREPQVYTLPPSQEEMTKNQVSLTCLVKGFYPSDIAVEWESNGQPENNYKTTPPVLDSDGSFFLYSRLTVDKSRWQEGNVFSCSVMHEALHNHYTQKSLSLSLGK

SEQ ID NO: 84 - protein, 214 aa, synthetic construct
DIQMTQSPSSLSASVGDRVTITCRASQDISNYLNWYQQKPGKAPKLLIYYKSRLHSGVPSRFSGSGSGTDFTFTISSLQPEDIATYYCQQVHTLPPTFGQGTKLEIKRTVAAPSVFIFPPSDEQLKSGTASVVCLLNNFYPREAKVQWKVDNALQSGNSQESVTEQDSKDSTYSLSSTLTLSKADYEKHKVYACEVTHQGLSSPVTKSFNRGEC

SEQ ID NO: 85 - protein, 214 aa, synthetic construct
DIQMTQSPSSLSASVGDRVTITCRASQDISNYLNWYQQKPGKAPKLLIYYKSRLHSGVPSRFSGSGSGTDFTLTISSLQPEDFATYYCQQVHTLPPTFGQGTKLEIKRTVAAPSVFIFPPSDEQLKSGTASVVCLLNNFYPREAKVQWKVDNALQSGNSQESVTEQDSKDSTYSLSSTLTLSKADYEKHKVYACEVTHQGLSSPVTKSFNRGEC

SEQ ID NO: 86 - protein, 214 aa, synthetic construct
EIVMTQSPPTLSLSPGERVTLSCRASQDISNYLNWYQQKPGQAPRLLIYYKSRLHSGIPARFSGSGSGTDFTLTISSLQPEDFAVYYCQQVHTLPPTFGQGTKLEIKRTVAAPSVFIFPPSDEQLKSGTASVVCLLNNFYPREAKVQWKVDNALQSGNSQESVTEQDSKDSTYSLSSTLTLSKADYEKHKVYACEVTHQGLSSPVTKSFNRGEC

SEQ ID NO: 87 - protein, 214 aa, synthetic construct
DIQMTQSPSSLSASVGDRVTITCRASQDISNYLNWYQQKPGKAPKLLIYYKSRLHSGVPSRFSGSGSGTDFTFTISSLQPEDIATYFCQQVHTLPPTFGQGTKLEIKRTVAAPSVFIFPPSDEQLKSGTASVVCLLNNFYPREAKVQWKVDNALQSGNSQESVTEQDSKDSTYSLSSTLTLSKADYEKHKVYACEVTHQGLSSPVTKSFNRGEC

SEQ ID NO: 88 - protein, 444 aa, synthetic construct
EVQLLQSAAEVKRPGESLRISCKTSGYSFTENTMHWVRQMPGKELEWMGGINPHKGGTSYNQKFKGHVTISVDKSSSTAYLQWSSLKASDAAMYYCARDWLGAMDYWGQGTLVTVSSASTKGPSVFPLAPCSRSTSESTAALGCLVKDYFPEPVTVSWNSGALTSGVHTFPAVLQSSGLYSLSSVVTVPSSSLGTKTYTCNVDHKPSNTKVDKRVESKYGPPCPPCPAPEFLGGPSVFLFPPKPKDTLMISRTPEVTCVVVDVSQEDPEVQFNWYVDGVEVHNAKTKPREEQFNSTYRVVSVLTVLHQDWLNGKEYKCKVSNKGLPSSIEKTISKAKGQPREPQVYTLPPSQEEMTKNQVSLTCLVKGFYPSDIAVEWESNGQPENNYKTTPPVLDSDGSFFLYSRLTVDKSRWQEGNVFSCSVMHEALHNHYTQKSLSLSLGK

SEQ ID NO: 89 - protein, 444 aa, synthetic construct
EVQLLQSAAEVKRPGESLRISCKTSGYTFTENTMHWVRQMPGKELEWMGGINPHKGGTSYNQKFKGHVTISADKSSSTAYLQWSSLKASDAAMYYCARDWLGAMDYWGQGTLVTVSSASTKGPSVFPLAPCSRSTSESTAALGCLVKDYFPEPVTVSWNSGALTSGVHTFPAVLQSSGLYSLSSVVTVPSSSLGTKTYTCNVDHKPSNTKVDKRVESKYGPPCPPCPAPEFLGGPSVFLFPPKPKDTLMISRTPEVTCVVVDVSQEDPEVQFNWYVDGVEVHNAKTKPREEQFNSTYRVVSVLTVLHQDWLNGKEYKCKVSNKGLPSSIEKTISKAKGQPREPQVYTLPPSQEEMTKNQVSLTCLVKGFYPSDIAVEWESNGQPENNYKTTPPVLDSDGSFFLYSRLTVDKSRWQEGNVFSCSVMHEALHNHYTQKSLSLSLGK

SEQ ID NO: 90 - protein, 444 aa, synthetic construct
EVQLLQSAAEVKRPGESLRISCKTSGYTFTENTMHWVRQMPGKELEWMGGINPHKGGTSYNQKFKGHVTLSVDKSSSTAYLQWSSLKASDAAMYYCARDWLGAMDYWGQGTLVTVSSASTKGPSVFPLAPCSRSTSESTAALGCLVKDYFPEPVTVSWNSGALTSGVHTFPAVLQSSGLYSLSSVVTVPSSSLGTKTYTCNVDHKPSNTKVDKRVESKYGPPCPPCPAPEFLGGPSVFLFPPKPKDTLMISRTPEVTCVVVDVSQEDPEVQFNWYVDGVEVHNAKTKPREEQFNSTYRVVSVLTVLHQDWLNGKEYKCKVSNKGLPSSIEKTISKAKGQPREPQVYTLPPSQEEMTKNQVSLTCLVKGFYPSDIAVEWESNGQPENNYKTTPPVLDSDGSFFLYSRLTVDKSRWQEGNVFSCSVMHEALHNHYTQKSLSLSLGK

SEQ ID NO: 91 - protein, 444 aa, synthetic construct
QVQLVQSGAEVKKPGASVKVSCKASGYTFTENTMHWVRQAPGQGLEWMGGINPHKGGTSYNQKFKGRVTLTVDKSSSTAYMELSRLRSDDTAVYYCARDWLGAMDYWGQGTLVTVSSASTKGPSVFPLAPCSRSTSESTAALGCLVKDYFPEPVTVSWNSGALTSGVHTFPAVLQSSGLYSLSSVVTVPSSSLGTKTYTCNVDHKPSNTKVDKRVESKYGPPCPPCPAPEFLGGPSVFLFPPKPKDTLMISRTPEVTCVVVDVSQEDPEVQFNWYVDGVEVHNAKTKPREEQFNSTYRVVSVLTVLHQDWLNGKEYKCKVSNKGLPSSIEKTISKAKGQPREPQVYTLPPSQEEMTKNQVSLTCLVKGFYPSDIAVEWESNGQPENNYKTTPPVLDSDGSFFLYSRLTVDKSRWQEGNVFSCSVMHEALHNHYTQKSLSLSLGK

SEQ ID NO: 92 - protein, 444 aa, synthetic construct
QVQLVQSGAEVKKPGSSVKVSCKASGYTFTENTMHWVRQAPGQGLEWMGGINPHKGGTSYNQKFKGRVTITVDKSTSTAYMELSSLRSEDTAVYYCARDWLGAMDYWGQGTLVTVSSASTKGPSVFPLAPCSRSTSESTAALGCLVKDYFPEPVTVSWNSGALTSGVHTFPAVLQSSGLYSLSSVVTVPSSSLGTKTYTCNVDHKPSNTKVDKRVESKYGPPCPPCPAPEFLGGPSVFLFPPKPKDTLMISRTPEVTCVVVDVSQEDPEVQFNWYVDGVEVHNAKTKPREEQFNSTYRVVSVLTVLHQDWLNGKEYKCKVSNKGLPSSIEKTISKAKGQPREPQVYTLPPSQEEMTKNQVSLTCLVKGFYPSDIAVEWESNGQPENNYKTTPPVLDSDGSFFLYSRLTVDKSRWQEGNVFSCSVMHEALHNHYTQKSLSLSLGK

SEQ ID NO: 93 - protein, 214 aa, synthetic construct
DIQLTQSPSSLSASVGDRVTITCITSTDIDDDMNWYRQKPGKVPKLLISEGNTLRPGVPSRFSGSGSGTDFTLTISSLQPEDVATYYCLQSDNLPYTFGQGTKLEIKRTVAAPSVFIFPPSDEQLKSGTASVVCLLNNFYPREAKVQWKVDNALQSGNSQESVTEQDSKDSTYSLSSTLTLSKADYEKHKVYACEVTHQGLSSPVTKSFNRGEC

SEQ ID NO: 94 - protein, 214 aa, synthetic construct
DIQVTQSPSSLSASVGDRVTITCITSTDIDDDMNWYQQKPGKAPKLLISEGNTLRPGVPSRFSGSGSGTDFTFTISSLQPEDIATYYCLQSDNLPYTFGQGTKLEIKRTVAAPSVFIFPPSDEQLKSGTASVVCLLNNFYPREAKVQWKVDNALQSGNSQESVTEQDSKDSTYSLSSTLTLSKADYEKHKVYACEVTHQGLSSPVTKSFNRGEC

SEQ ID NO: 95 - protein, 214 aa, synthetic construct
DIVLTQSPASLAVSPGQRATITCITSTDIDDDMNWYQQKPGQPPKLLISEGNTLRPGVPARFSSSGSGTDFTLTINPVEANDTANYYCLQSDNLPYTFGQGTKLEIKRTVAAPSVFIFPPSDEQLKSGTASVVCLLNNFYPREAKVQWKVDNALQSGNSQESVTEQDSKDSTYSLSSTLTLSKADYEKHKVYACEVTHQGLSSPVTKSFNRGEC

SEQ ID NO: 96 - protein, 214 aa, synthetic construct
DTVLTQSPASLAVSPGQRATITCITSTDIDDDMNWYQQKPGQPPKLLISEGNTLRPGVPARFSSSGSGTDFTLTINPVEANDTANYYCLQSDNLPYTFGQGTKLEIKRTVAAPSVFIFPPSDEQLKSGTASVVCLLNNFYPREAKVQWKVDNALQSGNSQESVTEQDSKDSTYSLSSTLTLSKADYEKHKVYACEVTHQGLSSPVTKSFNRGEC

SEQ ID NO: 97 - protein, 214 aa, synthetic construct
DIVLTQSPASLAVSPGQRATITCITSTDIDDDMNWYQQKPGQPPKLLISEGNTLRPGVPARFSSSGSGTDFTLTINPVEANDVANYYCLQSDNLPYTFGQGTKLEIKRTVAAPSVFIFPPSDEQLKSGTASVVCLLNNFYPREAKVQWKVDNALQSGNSQESVTEQDSKDSTYSLSSTLTLSKADYEKHKVYACEVTHQGLSSPVTKSFNRGEC

SEQ ID NO: 98 - protein, 444 aa, synthetic construct
QVQLVQSGAEVKKPGASVKVSCKASGYTFTSYNMLWVRQAPGQRLEWMGVIFPGNGDTSYNPKFKGRVTITADKSSSTAYMELSSLRSEDTAVYYCARDGYPSMDYWGQGTLVTVSSASTKGPSVFPLAPCSRSTSESTAALGCLVKDYFPEPVTVSWNSGALTSGVHTFPAVLQSSGLYSLSSVVTVPSSSLGTKTYTCNVDHKPSNTKVDKRVESKYGPPCPPCPAPEFLGGPSVFLFPPKPKDTLMISRTPEVTCVVVDVSQEDPEVQFNWYVDGVEVHNAKTKPREEQFNSTYRVVSVLTVLHQDWLNGKEYKCKVSNKGLPSSIEKTISKAKGQPREPQVYTLPPSQEEMTKNQVSLTCLVKGFYPSDIAVEWESNGQPENNYKTTPPVLDSDGSFFLYSRLTVDKSRWQEGNVFSCSVMHEALHNHYTQKSLSLSLGK

SEQ ID NO: 99 - protein, 444 aa, synthetic construct
QVQLVQSGAEVKKPGASVKVSCKASGYTFTSYNMLWVRQAPGQRLEWMGVIFPGNGDTSYNPKFKGRVTLTADKSSSTAYMELSSLRSEDTAVYYCARDGYPSMDYWGQGTLVTVSSASTKGPSVFPLAPCSRSTSESTAALGCLVKDYFPEPVTVSWNSGALTSGVHTFPAVLQSSGLYSLSSVVTVPSSSLGTKTYTCNVDHKPSNTKVDKRVESKYGPPCPPCPAPEFLGGPSVFLFPPKPKDTLMISRTPEVTCVVVDVSQEDPEVQFNWYVDGVEVHNAKTKPREEQFNSTYRVVSVLTVLHQDWLNGKEYKCKVSNKGLPSSIEKTISKAKGQPREPQVYTLPPSQEEMTKNQVSLTCLVKGFYPSDIAVEWESNGQPENNYKTTPPVLDSDGSFFLYSRLTVDKSRWQEGNVFSCSVMHEALHNHYTQKSLSLSLGK

SEQ ID NO: 100 - protein, 444 aa, synthetic construct
QVQLVQSGAEVKKPGSSVKVSCKASGYTFSSYNMLWVRQAPGQGLEWMGVIFPGNGDTSYNPKFKGRVTITADKSTSTAYMELSSLRSEDTAVYYCARDGYPSMDYWGQGTLVTVSSASTKGPSVFPLAPCSRSTSESTAALGCLVKDYFPEPVTVSWNSGALTSGVHTFPAVLQSSGLYSLSSVVTVPSSSLGTKTYTCNVDHKPSNTKVDKRVESKYGPPCPPCPAPEFLGGPSVFLFPPKPKDTLMISRTPEVTCVVVDVSQEDPEVQFNWYVDGVEVHNAKTKPREEQFNSTYRVVSVLTVLHQDWLNGKEYKCKVSNKGLPSSIEKTISKAKGQPREPQVYTLPPSQEEMTKNQVSLTCLVKGFYPSDIAVEWESNGQPENNYKTTPPVLDSDGSFFLYSRLTVDKSRWQEGNVFSCSVMHEALHNHYTQKSLSLSLGK

SEQ ID NO: 101 - protein, 444 aa, synthetic construct
QVQLVQSGAEVKKPGSSVKVSCKASGYTFTSYNMLWVRQAPGQGLEWMGVIFPGNGDTSYNPKFKGRVTITADKSTSTAYMELSSLRSEDTAVYYCARDGYPSMDYWGQGTLVTVSSASTKGPSVFPLAPCSRSTSESTAALGCLVKDYFPEPVTVSWNSGALTSGVHTFPAVLQSSGLYSLSSVVTVPSSSLGTKTYTCNVDHKPSNTKVDKRVESKYGPPCPPCPAPEFLGGPSVFLFPPKPKDTLMISRTPEVTCVVVDVSQEDPEVQFNWYVDGVEVHNAKTKPREEQFNSTYRVVSVLTVLHQDWLNGKEYKCKVSNKGLPSSIEKTISKAKGQPREPQVYTLPPSQEEMTKNQVSLTCLVKGFYPSDIAVEWESNGQPENNYKTTPPVLDSDGSFFLYSRLTVDKSRWQEGNVFSCSVMHEALHNHYTQKSLSLSLGK

SEQ ID NO: 102 - protein, 444 aa, synthetic construct
QVQLVQSGAEVKKPGSSVKVSCKASGYTFTSYNMLWVRQAPGQGLEWMGVIFPGNGDTSYNPKFKGRVTLTADKSSSTAYMELSSLRSEDTAVYYCARDGYPSMDYWGQGTLVTVSSASTKGPSVFPLAPCSRSTSESTAALGCLVKDYFPEPVTVSWNSGALTSGVHTFPAVLQSSGLYSLSSVVTVPSSSLGTKTYTCNVDHKPSNTKVDKRVESKYGPPCPPCPAPEFLGGPSVFLFPPKPKDTLMISRTPEVTCVVVDVSQEDPEVQFNWYVDGVEVHNAKTKPREEQFNSTYRVVSVLTVLHQDWLNGKEYKCKVSNKGLPSSIEKTISKAKGQPREPQVYTLPPSQEEMTKNQVSLTCLVKGFYPSDIAVEWESNGQPENNYKTTPPVLDSDGSFFLYSRLTVDKSRWQEGNVFSCSVMHEALHNHYTQKSLSLSLGK

SEQ ID NO: 103 - protein, 444 aa, synthetic construct
QVQLVQSGAEVKKPGASVKVSCKASGYTFTSYNMLWVRQAPGQRLEWMGVIFPGNADTSYNPKFKGRVTLTADKSSSTAYMELSSLRSEDTAVYYCARDGYPSMDYWGQGTLVTVSSASTKGPSVFPLAPCSRSTSESTAALGCLVKDYFPEPVTVSWNSGALTSGVHTFPAVLQSSGLYSLSSVVTVPSSSLGTKTYTCNVDHKPSNTKVDKRVESKYGPPCPPCPAPEFLGGPSVFLFPPKPKDTLMISRTPEVTCVVVDVSQEDPEVQFNWYVDGVEVHNAKTKPREEQFNSTYRVVSVLTVLHQDWLNGKEYKCKVSNKGLPSSIEKTISKAKGQPREPQVYTLPPSQEEMTKNQVSLTCLVKGFYPSDIAVEWESNGQPENNYKTTPPVLDSDGSFFLYSRLTVDKSRWQEGNVFSCSVMHEALHNHYTQKSLSLSLGK

SEQ ID NO: 104 - protein, 214 aa, synthetic construct
DIQMTQSPSSVSASVGDRVTITCITSTDIDDDMNWYQQKPGKAPKLLISEGNSLRPGVPSRFSGSGSGTDFTLTISSLQPEDFATYYCLQFNNMPLTFGQGTKLEIKRTVAAPSVFIFPPSDEQLKSGTASVVCLLNNFYPREAKVQWKVDNALQSGNSQESVTEQDSKDSTYSLSSTLTLSKADYEKHKVYACEVTHQGLSSPVTKSFNRGEC

SEQ ID NO: 105 - protein, 214 aa, synthetic construct
DIQLTQSPSFLSASVGDRVTITCITSTDIDDDMNWYQQKPGKAPKLLISEGNSLRPGVPSRFSSSGSGTEFTLTISSLQPEDFATYYCLQFNNMPLTFGQGTKLEIKRTVAAPSVFIFPPSDEQLKSGTASVVCLLNNFYPREAKVQWKVDNALQSGNSQESVTEQDSKDSTYSLSSTLTLSKADYEKHKVYACEVTHQGLSSPVTKSFNRGEC

SEQ ID NO: 106 - protein, 214 aa, synthetic construct
DTQLTQSPSFLSASVGDRVTITCITSTDIDDDMNWYQQKPGKAPKLLISEGNSLRPGVPSRFSSSGSGTEFTLTISSLQPEDFATYYCLQFNNMPLTFGQGTKLEIKRTVAAPSVFIFPPSDEQLKSGTASVVCLLNNFYPREAKVQWKVDNALQSGNSQESVTEQDSKDSTYSLSSTLTLSKADYEKHKVYACEVTHQGLSSPVTKSFNRGEC

SEQ ID NO: 107 - protein, 214 aa, synthetic construct
EIVLTQSPDFQSVTPKEKVTITCITSTDIDDDMNWYQQKPDQSPKLLISEGNSLRPGVPSRFSSSGSGTDFTLTINSLEAEDAATYYCLQFNNMPLTFGQGTKLEIKRTVAAPSVFIFPPSDEQLKSGTASVVCLLNNFYPREAKVQWKVDNALQSGNSQESVTEQDSKDSTYSLSSTLTLSKADYEKHKVYACEVTHQGLSSPVTKSFNRGEC

SEQ ID NO: 108 - protein, 445 aa, synthetic construct
EVQLVESGGGLVQPGGSLRLSCAASGFTFSSYTMSWVRQAPGKGLEWVATISGGGFGTYYPDSVKGRFTISRDNAKNSLYLQMNSLRAEDTAVYYCARPGYNNYYFDIWGQGTTVTVSSASTKGPSVFPLAPCSRSTSESTAALGCLVKDYFPEPVTVSWNSGALTSGVHTFPAVLQSSGLYSLSSVVTVPSSSLGTKTYTCNVDHKPSNTKVDKRVESKYGPPCPPCPAPEAAGGPSVFLFPPKPKDTLMISRTPEVTCVVVDVSQEDPEVQFNWYVDGVEVHNAKTKPREEQFNSTYRVVSVLTVLHQDWLNGKEYKCKVSNKGLPSSIEKTISKAKGQPREPQVYTLPPSQEEMTKNQVSLTCLVKGFYPSDIAVEWESNGQPENNYKTTPPVLDSDGSFFLYSRLTVDKSRWQEGNVFSCSVMHEALHNHYTQKSLSLSLG

SEQ ID NO: 109 - protein, 214 aa, synthetic construct
EIVLTQSPATLSLSPGERATLSCHASDSISNSLHWYQQKPGQAPRLLIYYARQSIQGIPARFSGSGSGTDFTLTISSLEPEDFAVYYCQQSESWPLHFGGGTKVEIKRTVAAPSVFIFPPSDEQLKSGTASVVCLLNNFYPREAKVQWKVDNALQSGNSQESVTEQDSKDSTYSLSSTLTLSKADYEKHKVYACEVTHQGLSSPVTKSFNRGEC

SEQ ID NO: 110 - protein, 446 aa, synthetic construct
QVQLVESGGGLVQPGGSLRLSCAASGFTFSSYWMSWVRQAPGKGLEWVSGISYSGSNTHYADSVKGRFTISRDNSKNTLYLQMNSLRAEDTAVYYCARMGIDLDYWGQGTLVTVSSASTKGPSVFPLAPSSKSTSGGTAALGCLVKDYFPEPVTVSWNSGALTSGVHTFPAVLQSSGLYSLSSVVTVPSSSLGTQTYICNVNHKPSNTKVDKRVEPKSCDKTHTCPPCPAPELLGGPSVFLFPPKPKDTLMISRTPEVTCVVVDVSHEDPEVKFNWYVDGVEVHNAKTKPREEQYNSTYRVVSVLTVLHQDWLNGKEYKCKVSNKALPAPIEKTISKAKGQPREPQVYTLPPSREEMTKNQVSLTCLVKGFYPSDIAVEWESNGQPENNYKTTPPVLDSDGSFFLYSKLTVDKSRWQQGNVFSCSVMHEALHNHYTQKSLSLSPGK

SEQ ID NO: 111 - protein, 217 aa, synthetic construct
DIALTQPASVSGSPGQSITISCTGTSSDVGGFNYVSWYQQHPGKAPKLMIHDGSNRPSGVSNRFSGSKSGNTASLTISGLQAEDEADYYCQSWDVSPITAVFGGGTKLTVLGQPKAAPSVTLFPPSSEELQANKATLVCLISDFYPGAVTVAWKADSSPVKAGVETTTPSKQSNNKYAASSYLSLTPEQWKSHRSYSCQVTHEGSTVEKTVAPTECS

SEQ ID NO: 112 - protein, 327 aa, synthetic construct
ASTKGPSVFPLAPCSRSTSESTAALGCLVKDYFPEPVTVSWNSGALTSGVHTFPAVLQSSGLYSLSSVVTVPSSSLGTKTYTCNVDHKPSNTKVDKRVESKYGPPCPPCPAPEFLGGPSVFLFPPKPKDTLMISRTPEVTCVVVDVSQEDPEVQFNWYVDGVEVHNAKTKPREEQFNSTYRVVSVLTVLHQDWLNGKEYKCKVSNKGLPSSIEKTISKAKGQPREPQVYTLPPSQEEMTKNQVSLTCLVKGFYPSDIAVEWESNGQPENNYKTTPPVLDSDGSFFLYSRLTVDKSRWQEGNVFSCSVMHEALHNHYTQKSLSLSLGK

SEQ ID NO: 113 - protein, 107 aa, synthetic construct [sequence omitted]